European Patent Application EP 4 541 890 A1, published April 23, 2025. Title: Methods for detecting fluorescence. Applicant: TOPPAN PRINTING CO., LTD. The sequence listing filed with the application follows.

SEQUENCE LISTING (49 sequences)

SEQ ID NO: 1 - DNA, 35 bp, synthetic construct
  source 1..35: mol_type = other DNA
  misc_feature 1: note = Modified with Alexa Fluor 488
  misc_feature 5: note = Modified with BHQ-1
ttcttagccggttttccggctgagacctcggcgcg

SEQ ID NO: 2 - DNA, 35 bp, synthetic construct
  source 1..35: mol_type = other DNA
  misc_feature 1: note = Modified with ATTO 542
  misc_feature 5: note = Modified with BHQ-1
ttcttagccggttttccggctgagacggcctcgcg

SEQ ID NO: 3 - DNA, 37 bp, synthetic construct
  source 1..37: mol_type = other DNA
  misc_feature 1: note = Modified with Alexa Fluor 568
  misc_feature 5: note = Modified with BHQ-2
ttcttagccggttttccggctgagactccgcgtccgt

SEQ ID NO: 4 - DNA, 38 bp, synthetic construct
  source 1..38: mol_type = other DNA
  misc_feature 1: note = Modified with ATTO 643
  misc_feature 5: note = Modified with BHQ-2
ttcttagccggttttccggctgagacgatgcgagctca

SEQ ID NO: 5 - DNA, 38 bp, synthetic construct; identical to SEQ ID NO: 4
  source 1..38: mol_type = other DNA
  misc_feature 1: note = Modified with ATTO 643
  misc_feature 5: note = Modified with BHQ-1

SEQ ID NO: 6 - DNA, 38 bp, synthetic construct; identical to SEQ ID NO: 4
  source 1..38: mol_type = other DNA
  misc_feature 1: note = Modified with ATTO 643
  misc_feature 5: note = Modified with BHQ-3

SEQ ID NO: 7 - DNA, 101 bp, synthetic construct
  source 1..101: mol_type = other DNA
ctttgtgttcccggacatagtccaggaggcagccgaagggcatgagctgcgtgatgagctgcacggtggaggtgaggcagatgcccagcaggcggcacacg

SEQ ID NO: 8 - DNA, 101 bp, synthetic construct
  source 1..101: mol_type = other DNA
ctttgtgttcccggacatagtccaggaggcagccgaagggcatgagctgcatgatgagctgcacggtggaggtgaggcagatgcccagcaggcggcacacg

SEQ ID NO: 9 - DNA, 101 bp, synthetic construct
  source 1..101: mol_type = other DNA
gccaggaacgtactggtgaaaacaccgcagcatgtcaagatcacagattttgggctggccaaactgctgggtgcggaagagaaagaataccatgcagaagg

SEQ ID NO: 10 - DNA, 101 bp, synthetic construct
  source 1..101: mol_type = other DNA
gccaggaacgtactggtgaaaacaccgcagcatgtcaagatcacagattttgggcgggccaaactgctgggtgcggaagagaaagaataccatgcagaagg

SEQ ID NO: 11 - DNA, 24 bp, synthetic construct
  source 1..24: mol_type = other DNA
cgcgccgaggcgcagctcatgccc

SEQ ID NO: 12 - DNA, 26 bp, synthetic construct
  source 1..26: mol_type = other DNA
acggacgcggagtgcagctcatgccc

SEQ ID NO: 13 - DNA, 31 bp, synthetic construct
  source 1..31: mol_type = other DNA
tctgcctcacctccaccgtgcarctcatcaa

SEQ ID NO: 14 - DNA, 30 bp, synthetic construct
  source 1..30: mol_type = other DNA
cgcgaggccgagcccaaaatctgtgatctt

SEQ ID NO: 15 - DNA, 33 bp, synthetic construct
  source 1..33: mol_type = other DNA
tgagctcgcatcgcgcccaaaatctgtgatctt

SEQ ID NO: 16 - DNA, 20 bp, synthetic construct
  source 1..20: mol_type = other DNA
cgcacccagcagtttggcca

SEQ ID NO: 17 - DNA, 105 bp, synthetic construct
  source 1..105: mol_type = other DNA
ccgaagggcatgagctgcgtgatgagctgcacggtggaggtgaggcagatgcccagcaggcggcacacgtgggggttgtccacgctggccatcacgtaggcttcc

SEQ ID NO: 18 - DNA, 24 bp, synthetic construct
  source 1..24: mol_type = other DNA
cgcgccgaggcgcagctcatgccc

SEQ ID NO: 19 - DNA, 19 bp, synthetic construct
  source 1..19: mol_type = other DNA
ccaccgtgcagctcatcaa

SEQ ID NO: 20 - DNA, 11 bp, synthetic construct
  source 1..11: mol_type = other DNA
cgcgccgaggc

SEQ ID NO: 21 - DNA, 34 bp, synthetic construct
  source 1..34: mol_type = other DNA
  misc_feature 1: note = Modified with fluorescein
  misc_feature 4: note = Modified with BHQ-1
tcttagccggttttccggctgagacctcggcgcg

SEQ ID NO: 22 - DNA, 34 bp, synthetic construct; identical to SEQ ID NO: 21
  source 1..34: mol_type = other DNA
  misc_feature 1: note = Modified with fluorescein
  misc_feature 4: note = Modified with BHQ-1

SEQ ID NO: 23 - DNA, 105 bp, synthetic construct; identical to SEQ ID NO: 17
  source 1..105: mol_type = other DNA

SEQ ID NO: 24 - DNA, 24 bp, synthetic construct
  source 1..24: mol_type = other DNA
cgcgccgaggcgcagctcatgccc

SEQ ID NO: 25 - DNA, 19 bp, synthetic construct
  source 1..19: mol_type = other DNA
ccaccgtgcagctcatcaa

SEQ ID NO: 26 - DNA, 11 bp, synthetic construct
  source 1..11: mol_type = other DNA
cgcgccgaggc

SEQ ID NO: 27 - DNA, 34 bp, synthetic construct; identical to SEQ ID NO: 21
  source 1..34: mol_type = other DNA
  misc_feature 1: note = Modified with fluorescein
  misc_feature 4: note = Modified with BHQ-1

SEQ ID NO: 28 - DNA, 34 bp, synthetic construct; identical to SEQ ID NO: 21
  source 1..34: mol_type = other DNA
  misc_feature 1: note = Modified with fluorescein
  misc_feature 4: note = Modofied with BHQ-1

SEQ ID NO: 29 - DNA, 33 bp, synthetic construct
  source 1..33: mol_type = other DNA
  misc_feature 1: note = Modified with fluorescein
tctagccggttttccggctgagacctcggcgcg

SEQ ID NO: 30 - DNA, 34 bp, synthetic construct; identical to SEQ ID NO: 21
  source 1..34: mol_type = other DNA
  misc_feature 1: note = Modified with fluorescein
  misc_feature 4: note = Modified with BHQ-1

SEQ ID NO: 31 - DNA, 35 bp, synthetic construct; identical to SEQ ID NO: 1
  source 1..35: mol_type = other DNA
  misc_feature 1: note = Modified with BHQ-1
  misc_feature 5: note = Modified with fluorescein

SEQ ID NO: 32 - DNA, 34 bp, synthetic construct; identical to SEQ ID NO: 21
  source 1..34: mol_type = other DNA
  misc_feature 1: note = Modified with fluorescein
  misc_feature 4: note = Modified with BHQ-1

SEQ ID NO: 33 - DNA, 34 bp, synthetic construct
  source 1..34: mol_type = other DNA
  misc_feature 1: note = Modified with fluorescein
  misc_feature 21: note = Modified with BHQ-1
tctgagccggttttccggcttagacctcggcgcg

SEQ ID NO: 34 - DNA, 34 bp, synthetic construct; identical to SEQ ID NO: 21
  source 1..34: mol_type = other DNA
  misc_feature 1: note = Modified with fluorescein
  misc_feature 4: note = Modified with BHQ-1

SEQ ID NO: 35 - DNA, 34 bp, synthetic construct; identical to SEQ ID NO: 21
  source 1..34: mol_type = other DNA
  misc_feature 1: note = Modified with fluorescent substance
  misc_feature 4: note = Modified with Quencher

SEQ ID NO: 36 - DNA, 105 bp, synthetic construct; identical to SEQ ID NO: 17
  source 1..105: mol_type = other DNA

SEQ ID NO: 37 - DNA, 24 bp, synthetic construct
  source 1..24: mol_type = other DNA
cgcgccgaggcgcagctcatgccc

SEQ ID NO: 38 - DNA, 19 bp, synthetic construct
  source 1..19: mol_type = other DNA
ccaccgtgcagctcatcaa

SEQ ID NO: 39 - DNA, 11 bp, synthetic construct
  source 1..11: mol_type = other DNA
cgcgccgaggc

SEQ ID NO: 40 - DNA, 33 bp, synthetic construct
  source 1..33: mol_type = other DNA
  misc_feature 1: note = Modified with fluorescein
  misc_feature 4: note = Modified with BHQ-1
tcttagccggttttccggctagacctcggcgcg

SEQ ID NO: 41 - DNA, 34 bp, synthetic construct; identical to SEQ ID NO: 21
  source 1..34: mol_type = other DNA
  misc_feature 1: note = Modified with fluorescein
  misc_feature 4: note = Modified with BHQ-1

SEQ ID NO: 42 - DNA, 105 bp, synthetic construct; identical to SEQ ID NO: 17
  source 1..105: mol_type = other DNA

SEQ ID NO: 43 - DNA, 24 bp, synthetic construct
  source 1..24: mol_type = other DNA
cgcgccgaggcgcagctcatgccc

SEQ ID NO: 44 - DNA, 19 bp, synthetic construct
  source 1..19: mol_type = other DNA
ccaccgtgcagctcatcaa

SEQ ID NO: 45 - DNA, 11 bp, synthetic construct
  source 1..11: mol_type = other DNA
cgcgccgaggc

SEQ ID NO: 46 - DNA, 33 bp, synthetic construct
  source 1..33: mol_type = other DNA
  misc_feature 1: note = Modified with fluorescein
  misc_feature 3: note = Modified with BHQ-1
cttagccggttttccggctgagacctcggcgcg

SEQ ID NO: 47 - DNA, 34 bp, synthetic construct; identical to SEQ ID NO: 21
  source 1..34: mol_type = other DNA
  misc_feature 1: note = Modified with fluorescein
  misc_feature 4: note = Modified with BHQ-1

SEQ ID NO: 48 - DNA, 35 bp, synthetic construct; identical to SEQ ID NO: 1
  source 1..35: mol_type = other DNA
  misc_feature 1: note = Modified with fluorescein
  misc_feature 5: note = Modified with BHQ-1

SEQ ID NO: 49 - DNA, 36 bp, synthetic construct
  source 1..36: mol_type = other DNA
  misc_feature 1: note = Modified with fluorescein
  misc_feature 6: note = Modified with BHQ-1
tttcttagccggttttccggctgagacctcggcgcg